European Patent Application EP 4 643 888 A1, published November 5, 2025. Title: ANTI-B7H3 AND PD-L1 BISPECIFIC ANTIBODY-DRUG CONJUGATE, PREPARATION METHOD THEREFOR, AND USE THEREOF. Applicant: DUALITY BIOLOGICS (SUZHOU) CO., LTD. The sequence listing filed with the application follows.

SEQUENCE LISTING (22 sequences)

SEQ ID NO: 1 - protein, 11 aa, synthetic construct
RASQSINTYLH

SEQ ID NO: 2 - protein, 7 aa, synthetic construct
YASQSIS

SEQ ID NO: 3 - protein, 9 aa, synthetic construct
QNGHSFPLT

SEQ ID NO: 4 - protein, 107 aa, synthetic construct
DIQMTQSPSSLSASVGDRVTISCRASQSINTYLHWYQQKLGQAPRLLIYYASQSISGVPSRFSGSGSGTDFTLTINSLEAEDAATYYCQNGHSFPLTFGAGTKVEIK

SEQ ID NO: 5 - protein, 5 aa, synthetic construct
TFGVH

SEQ ID NO: 6 - protein, 16 aa, synthetic construct
IIWPGGNTNYNSALMS

SEQ ID NO: 7 - protein, 9 aa, synthetic construct
ENYGRAMDY

SEQ ID NO: 8 - protein, 117 aa, synthetic construct
QVQLVQSGAEVKKPGASVKVSCKASGYTFTTFGVHWVRQAPGKGLEWVGIIWPGGNTNYNSALMSRVTITADESTSTAYMELSSLRSEDTAVYYCARENYGRAMDYWGQGTTVTVSS

SEQ ID NO: 9 - protein, 214 aa, synthetic construct
DIQMTQSPSSLSASVGDRVTISCRASQSINTYLHWYQQKLGQAPRLLIYYASQSISGVPSRFSGSGSGTDFTLTINSLEAEDAATYYCQNGHSFPLTFGAGTKVEIKRTVAAPSVFIFPPSDEQLKSGTASVVCLLNNFYPREAKVQWKVDNALQSGNSQESVTEQDSKDSTYSLSSTLTLSKADYEKHKVYACEVTHQGLSSPVTKSFNRGEC

SEQ ID NO: 10 - protein, 447 aa, synthetic construct
QVQLVQSGAEVKKPGASVKVSCKASGYTFTTFGVHWVRQAPGKGLEWVGIIWPGGNTNYNSALMSRVTITADESTSTAYMELSSLRSEDTAVYYCARENYGRAMDYWGQGTTVTVSSASTKGPSVFPLAPSSKSTSGGTAALGCLVKDYFPEPVTVSWNSGALTSGVHTFPAVLQSSGLYSLSSVVTVPSSSLGTQTYICNVNHKPSNTKVDKKVEPKSCDKTHTCPPCPAPELLGGPSVFLFPPKPKDTLMISRTPEVTCVVVDVSHEDPEVKFNWYVDGVEVHNAKTKPREEQYNSTYRVVSVLTVLHQDWLNGKEYKCKVSNKALPAPIEKTISKAKGQPREPQVYTLPPSREEMTKNQVSLTCLVKGFYPSDIAVEWESNGQPENNYKTTPPVLDSDGSFFLYSKLTVDKSRWQQGNVFSCSVMHEALHNHYTQKSLSLSPGK

SEQ ID NO: 11 - protein, 15 aa, synthetic construct
GGGGSGGGGTGGGGS

SEQ ID NO: 12 - protein, 5 aa, synthetic construct
TIWIG

SEQ ID NO: 13 - protein, 17 aa, synthetic construct
AIYIGSGATYYVDSVKG

SEQ ID NO: 14 - protein, 19 aa, synthetic construct
TGGTVGSMVRFSPVGDFGY

SEQ ID NO: 15 - protein, 128 aa, synthetic construct
DVQLQESGGGLVQAGGSLRLSCTASGYTLSTIWIGWFRQAPGKGLEGVAAIYIGSGATYYVDSVKGRFTISQDNAKNTVYLQMNSLKPEDTAMYYCAATGGTVGSMVRFSPVGDFGYWGQGTQVTVSS

SEQ ID NO: 16 - protein, 590 aa, synthetic construct
QVQLVQSGAEVKKPGASVKVSCKASGYTFTTFGVHWVRQAPGKGLEWVGIIWPGGNTNYNSALMSRVTITADESTSTAYMELSSLRSEDTAVYYCARENYGRAMDYWGQGTTVTVSSASTKGPSVFPLAPSSKSTSGGTAALGCLVKDYFPEPVTVSWNSGALTSGVHTFPAVLQSSGLYSLSSVVTVPSSSLGTQTYICNVNHKPSNTKVDKKVEPKSCDKTHTCPPCPAPELLGGPSVFLFPPKPKDTLMISRTPEVTCVVVDVSHEDPEVKFNWYVDGVEVHNAKTKPREEQYNSTYRVVSVLTVLHQDWLNGKEYKCKVSNKALPAPIEKTISKAKGQPREPQVYTLPPSREEMTKNQVSLTCLVKGFYPSDIAVEWESNGQPENNYKTTPPVLDSDGSFFLYSKLTVDKSRWQQGNVFSCSVMHEALHNHYTQKSLSLSPGKGGGGSGGGGTGGGGSDVQLQESGGGLVQAGGSLRLSCTASGYTLSTIWIGWFRQAPGKGLEGVAAIYIGSGATYYVDSVKGRFTISQDNAKNTVYLQMNSLKPEDTAMYYCAATGGTVGSMVRFSPVGDFGYWGQGTQVTVSS

SEQ ID NO: 17 - protein, 362 aa, synthetic construct
DVQLQESGGGLVQAGGSLRLSCTASGYTLSTIWIGWFRQAPGKGLEGVAAIYIGSGATYYVDSVKGRFTISQDNAKNTVYLQMNSLKPEDTAMYYCAATGGTVGSMVRFSPVGDFGYWGQGTQVTVSSGSEPKSCDKTHTCPPCPAPELLGGPSVFLFPPKPKDTLMISRTPEVTCVVVDVSHEDPEVKFNWYVDGVEVHNAKTKPREEQYNSTYRVVSVLTVLHQDWLNGKEYKCKVSNKALPAPIEKTISKAKGQPREPQVYTLPPSREEMTKNQVSLTCLVKGFYPSDIAVEWESNGQPENNYKTTPPVLDSDGSFFLYSKLTVDKSRWQQGNVFSCSVMHEALHNHYTQKSLSLSPGK

SEQ ID NO: 18 - protein, 600 aa, synthetic construct
QVQLVQSGAEVKKPGASVKVSCQASGYRFSNFVIHWVRQAPGQRFEWMGWINPYNGNKEFSAKFQDRVTFTADTSANTAYMELRSLRSADTAVYYCARVGPYSWDDSPQDNYYMDVWGKGTTVIVSSASTKGPSVFPLAPSSKSTSGGTAALGCLVKDYFPEPVTVSWNSGALTSGVHTFPAVLQSSGLYSLSSVVTVPSSSLGTQTYICNVNHKPSNTKVDKKVEPKSCDKTHTCPPCPAPELLGGPSVFLFPPKPKDTLMISRTPEVTCVVVDVSHEDPEVKFNWYVDGVEVHNAKTKPREEQYNSTYRVVSVLTVLHQDWLNGKEYKCKVSNKALPAPIEKTISKAKGQPREPQVYTLPPSREEMTKNQVSLTCLVKGFYPSDIAVEWESNGQPENNYKTTPPVLDSDGSFFLYSKLTVDKSRWQQGNVFSCSVMHEALHNHYTQKSLSLSPGKGGGGSGGGGTGGGGSDVQLQESGGGLVQAGGSLRLSCTASGYTLSTIWIGWFRQAPGKGLEGVAAIYIGSGATYYVDSVKGRFTISQDNAKNTVYLQMNSLKPEDTAMYYCAATGGTVGSMVRFSPVGDFGYWGQGTQVTVSS

SEQ ID NO: 19 - protein, 215 aa, synthetic construct
EIVLTQSPGTLSLSPGERATFSCRSSHSIRSRRVAWYQHKPGQAPRLVIHGVSNRASGISDRFSGSGSGTDFTLTITRVEPEDFALYYCQVYGASSYTFGQGTKLERKRTVAAPSVFIFPPSDEQLKSGTASVVCLLNNFYPREAKVQWKVDNALQSGNSQESVTEQDSKDSTYSLSSTLTLSKADYEKHKVYACEVTHQGLSSPVTKSFNRGEC

SEQ ID NO: 20 - protein, 447 aa, synthetic construct; identical to SEQ ID NO: 10

SEQ ID NO: 21 - protein, 447 aa, synthetic construct
QVQLVQSGVEVKKPGASVKVSCKASGYTFTNYYMYWVRQAPGQGLEWMGGINPSNGGTNFNEKFKNRVTLTTDSSTTTAYMELKSLQFDDTAVYYCARRDYRFDMGFDYWGQGTTVTVSSASTKGPSVFPLAPCSRSTSESTAALGCLVKDYFPEPVTVSWNSGALTSGVHTFPAVLQSSGLYSLSSVVTVPSSSLGTKTYTCNVDHKPSNTKVDKRVESKYGPPCPPCPAPEFLGGPSVFLFPPKPKDTLMISRTPEVTCVVVDVSQEDPEVQFNWYVDGVEVHNAKTKPREEQFNSTYRVVSVLTVLHQDWLNGKEYKCKVSNKGLPSSIEKTISKAKGQPREPQVYTLPPSQEEMTKNQVSLTCLVKGFYPSDIAVEWESNGQPENNYKTTPPVLDSDGSFFLYSRLTVDKSRWQEGNVFSCSVMHEALHNHYTQKSLSLSLGK

SEQ ID NO: 22 - protein, 218 aa, synthetic construct
EIVLTQSPATLSLSPGERATLSCRASKGVSTSGYSYLHWYQQKPGQAPRLLIYLASYLESGVPARFSGSGSGTDFTLTISSLEPEDFAVYYCQHSRDLPLTFGGGTKVEIKRTVAAPSVFIFPPSDEQLKSGTASVVCLLNNFYPREAKVQWKVDNALQSGNSQESVTEQDSKDSTYSLSSTLTLSKADYEKHKVYACEVTHQGLSSPVTKSFNRGEC